European Patent Application EP 4 455 161 A1, published October 30, 2024. Title: Human-derived anti-CRMP2 antibodies. Applicant: ONO PHARMACEUTICAL CO., LTD. Application EP. The sequence listing filed with the application follows.

SEQUENCE LISTING (72 sequences)

SEQ ID NO: 1 - DNA, 369 bp, Homo sapiens
  source 1..369: mol_type = other DNA
gaggtgcagctggtggagactgggggaggcttcgtccagccgggggggtccctacaactctcctgtgccgtctctggattcccctacagtggcacttctttccactgggtccgccaggtttccgggaaagggctggagtggattggccgtattagaagtaaaagtgacaattatgaaacatcatatactgagtcactgaagggcaggttcatcgtctccagagatgattcgaagaatatggtgcgtctgcacttgtacagtctgaggaccgaggacacggccctttattattgtactaccgggattatcgtggtggatacgtcgtatttggaccactggggccggggaaccctggtcaccgtctcctcg

SEQ ID NO: 2 - protein, 123 aa, Homo sapiens
EVQLVETGGGFVQPGGSLQLSCAVSGFPYSGTSFHWVRQVSGKGLEWIGRIRSKSDNYETSYTESLKGRFIVSRDDSKNMVRLHLYSLRTEDTALYYCTTGIIVVDTSYLDHWGRGTLVTVSS

SEQ ID NO: 3 - protein, 5 aa, Homo sapiens
GTSFH

SEQ ID NO: 4 - protein, 19 aa, Homo sapiens
RIRSKSDNYETSYTESLKG

SEQ ID NO: 5 - protein, 12 aa, Homo sapiens
GIIVVDTSYLDH

SEQ ID NO: 6 - DNA, 324 bp, Homo sapiens
  source 1..324: mol_type = other DNA
tcctatgagctgactcagccaccctcggcgtcagtgtccccaggacaaacggccaggatcacctgctctggagctgcattgccaaaaaaatatgcttattggtaccaactgaagtcaggccaggcccctgtgttggtcatctatgaagacactaaacggccctccgggatccctgagagattctctggctccagctcagggactttggccaccctgactatcaatggggccctcgtggaggatgaagctgactactactgttactcaacagacagcagtggtgatgtttgggtgttcggcggagggaccaagttgaccgtccta

SEQ ID NO: 7 - protein, 108 aa, Homo sapiens
SYELTQPPSASVSPGQTARITCSGAALPKKYAYWYQLKSGQAPVLVIYEDTKRPSGIPERFSGSSSGTLATLTINGALVEDEADYYCYSTDSSGDVWVFGGGTKLTVL

SEQ ID NO: 8 - protein, 11 aa, Homo sapiens
SGAALPKKYAY

SEQ ID NO: 9 - protein, 7 aa, Homo sapiens
EDTKRPS

SEQ ID NO: 10 - protein, 11 aa, Homo sapiens
YSTDSSGDVWV

SEQ ID NO: 11 - DNA, 369 bp, Homo sapiens
  source 1..369: mol_type = other DNA
gaagttcaactggtagagaccggagggggatttgtgcaaccgggggggagcttgcaactgagctgcgcggtatccggctttccatactcggggacctcttttcattgggtccgacaagtcagcggaaagggactggaatggattgggcgaatccgaagcaaaagcgacaactatgagacgagctacaccgagagcttgaagggacgattcatcgtgagcagggacgattctaagaatacggtaaggctgcacctaagcagcctgcgaaccgaagacaccgcgctatattactgcacgacggggatcattgtcgtcgacacctcatacttggaccactggggccgagggacgctagtgacggtctcgagc

SEQ ID NO: 12 - protein, 123 aa, Homo sapiens
EVQLVETGGGFVQPGGSLQLSCAVSGFPYSGTSFHWVRQVSGKGLEWIGRIRSKSDNYETSYTESLKGRFIVSRDDSKNTVRLHLSSLRTEDTALYYCTTGIIVVDTSYLDHWGRGTLVTVSS

SEQ ID NO: 13 - DNA, 369 bp, Homo sapiens
  source 1..369: mol_type = other DNA
gaagtgcaactggtggagaccggggggggatttgtacaaccgggggggagcctacagctgagctgcgcggtatcgggattcccatactccggcacgagctttcattgggtcaggcaatcgagcgggaaagggctggaatggatcgggaggattaggagcaagagcgacaactatgaaacatcatatacggagagcctgaagggaagattcatagtgagccgggatgactcaaagaacaccgtgcgactgcatctgagcagcttgcggactgaggatacggctctatactattgcacgacggggatcattgtcgtcgatacgagctacctggatcactgggggaggggaacactcgtgacggtctcgagc

SEQ ID NO: 14 - protein, 123 aa, Homo sapiens
EVQLVETGGGFVQPGGSLQLSCAVSGFPYSGTSFHWVRQSSGKGLEWIGRIRSKSDNYETSYTESLKGRFIVSRDDSKNTVRLHLSSLRTEDTALYYCTTGIIVVDTSYLDHWGRGTLVTVSS

SEQ ID NO: 15 - DNA, 369 bp, Homo sapiens
  source 1..369: mol_type = other DNA
gaggtgcaactggtagaaaccggggggggattcgtgcaaccgggggggagcttacaattaagctgcgcggtatcgggcttcccctatagcggaacatcattccattgggtccggcaagtctctgggaaggggctggaatggattggacggattcggagcaagagcgacaattacgagacatcatataccgaatcattaaaagggcgatttaccgtatcaagagacgattcgaaaaatacggtgcggctacacctatcatcgctgagaacggaggataccgcactatactattgcacaacggggataattgtcgtcgacacaagctacttggatcattgggggcgagggacacttgtgacggtctcgagc

SEQ ID NO: 16 - protein, 123 aa, Homo sapiens
EVQLVETGGGFVQPGGSLQLSCAVSGFPYSGTSFHWVRQVSGKGLEWIGRIRSKSDNYETSYTESLKGRFTVSRDDSKNTVRLHLSSLRTEDTALYYCTTGIIVVDTSYLDHWGRGTLVTVSS

SEQ ID NO: 17 - DNA, 369 bp, Homo sapiens
  source 1..369: mol_type = other DNA
gaggtgcaactggtggagaccgggggaggatttgtgcaacccggcgggagcctccaactgagctgcgcggtctccggcttcccatactctgggacgagcttccactgggtccggcaatcgagcgggaaaggcctggaatggatcggccggattagatcgaagagcgacaactatgaaacgagctatacggaatcactgaagggacgattcacggtatcgcgggatgactctaaaaataccgtgaggctacacctatcatccttgcggaccgaggacaccgcgctatattactgcacgacggggataattgtcgtcgatacgagctacttagaccattgggggagaggcaccttggtaacggtctcgagc

SEQ ID NO: 18 - protein, 123 aa, Homo sapiens
EVQLVETGGGFVQPGGSLQLSCAVSGFPYSGTSFHWVRQSSGKGLEWIGRIRSKSDNYETSYTESLKGRFTVSRDDSKNTVRLHLSSLRTEDTALYYCTTGIIVVDTSYLDHWGRGTLVTVSS

SEQ ID NO: 19 - DNA, 369 bp, Homo sapiens
  source 1..369: mol_type = other DNA
gaagtccaactggtcgagactggggggggctttgtgcaaccggggggatcgctgcaactatcatgcgccgtcagcggattcccatactctggaacatcatttcattgggtccgacaagcgagcggaaaggggctggaatggatcggacgcatacgatctaagagcgacaattacgaaacatcttatacggaatcgctcaaagggcgatttactgtgagccgggacgactcgaagaacacggtcaggctgcaccttagctcactgagaacggaagatacggcgctatactactgcactactgggatcatagtcgtcgatacgagctatctggaccactgggggaggggcacgctggtcacggtctcgagc

SEQ ID NO: 20 - protein, 123 aa, Homo sapiens
EVQLVETGGGFVQPGGSLQLSCAVSGFPYSGTSFHWVRQASGKGLEWIGRIRSKSDNYETSYTESLKGRFTVSRDDSKNTVRLHLSSLRTEDTALYYCTTGIIVVDTSYLDHWGRGTLVTVSS

SEQ ID NO: 21 - DNA, 369 bp, Homo sapiens
  source 1..369: mol_type = other DNA
gaggtgcaactggtggaatcggggggcggattcgtgcaaccgggcgggagcttgcgactatcatgcgcggttagcggatttccatatagcgggacatcatttcactgggtccggcaagcaagcggaaaagggctggaatggattggccgcattcggagcaaatccgacaactatgagacgagctatacggaatcattgaaaggaagattcacggtatcgagggatgactctaaaaacactgtatacctgcaactgagcagcttgcgaacggaagacaccgcgctatactactgcacgacggggatcatagtcgtcgatacctcatacctggaccactggggccggggaacactggtcacggtctcgagc

SEQ ID NO: 22 - protein, 123 aa, Homo sapiens
EVQLVESGGGFVQPGGSLRLSCAVSGFPYSGTSFHWVRQASGKGLEWIGRIRSKSDNYETSYTESLKGRFTVSRDDSKNTVYLQLSSLRTEDTALYYCTTGIIVVDTSYLDHWGRGTLVTVSS

SEQ ID NO: 23 - DNA, 369 bp, Homo sapiens
  source 1..369: mol_type = other DNA
gaggtgcaactggtggagaccggagggggatttgtgcaacctggaggatcactgcggctaagctgcgcggtatccggcttcccttatagcggaacatccttccactgggtccggcaagcatccggcaagggcttggaatggatcgggcggattagatcgaagagcgacaattacgaaacatcttataccgagagcctgaaggggagatttacggtaagcagggacgactcgaaaaatactgtatacctgcaactgagcagcctgaggaccgaagacacggccttatactactgcacaaccggcattatcgtcgtcgacactagctatctggatcattgggggcggggaacactcgtgacggtctcgagc

SEQ ID NO: 24 - protein, 123 aa, Homo sapiens
EVQLVETGGGFVQPGGSLRLSCAVSGFPYSGTSFHWVRQASGKGLEWIGRIRSKSDNYETSYTESLKGRFTVSRDDSKNTVYLQLSSLRTEDTALYYCTTGIIVVDTSYLDHWGRGTLVTVSS

SEQ ID NO: 25 - DNA, 369 bp, Homo sapiens
  source 1..369: mol_type = other DNA
gaagtgcaattagtggagagcgggggcggattcgtgcaaccgggggggagccttcaactgagctgcgctgtgagcggatttccttatagcggaacatcatttcattgggtccgacaagcctccgggaagggactggaatggatcgggaggattaggagcaaatccgacaattacgaaacaagctacactgaatccctgaagggccgatttaccgtgagccgagacgattcaaagaatacggtatacctgcaactatcatcactgcggactgaggataccgcgctatactactgcacaacggggataatagtcgtcgacacatcatacctcgaccattgggggagggggacgctggtcacggtctcgagc

SEQ ID NO: 26 - protein, 123 aa, Homo sapiens
EVQLVESGGGFVQPGGSLQLSCAVSGFPYSGTSFHWVRQASGKGLEWIGRIRSKSDNYETSYTESLKGRFTVSRDDSKNTVYLQLSSLRTEDTALYYCTTGIIVVDTSYLDHWGRGTLVTVSS

SEQ ID NO: 27 - DNA, 369 bp, Homo sapiens
  source 1..369: mol_type = other DNA
gaggtccaactggttgaaagcggagggggattcgtgcaacccggaggaagcctgagattgagctgcgccgtatcgggattcccatactcgggaacatcctttcactgggtccggcaagcaagcgggaagggccttgaatggattgggcgcattcgatcgaaatcggataactatgaaacgagctataccgaatcgctgaaggggcgattcacggttagcagagatgactccaaaaacacggtgcggctgcaactatcatcgctgcggaccgaggacaccgcgctatactattgcacgacggggataatcgtcgtcgacacgagctacctggaccactgggggaggggcacgctggtaacggtctcgagc

SEQ ID NO: 28 - protein, 123 aa, Homo sapiens
EVQLVESGGGFVQPGGSLRLSCAVSGFPYSGTSFHWVRQASGKGLEWIGRIRSKSDNYETSYTESLKGRFTVSRDDSKNTVRLQLSSLRTEDTALYYCTTGIIVVDTSYLDHWGRGTLVTVSS

SEQ ID NO: 29 - DNA, 369 bp, Homo sapiens
  source 1..369: mol_type = other DNA
gaggtccagctggtagagagcgggggcggcttcgtgcaaccgggaggatcgctgaggctgagctgcgccgtatcgggctttccttactccggcacttcattccactgggtccggcaagcatctgggaaagggcttgaatggatcgggcggatacggagcaaatccgacaattatgagacttcatatacggaatccctgaaggggagatttacggtatcgagggatgattcaaagaataccgtatatctgcacctgagctcgctgcgcacggaagacaccgcattatactactgcaccactggaatcattgtcgtcgatacaagctacttggatcattgggggagggggacgctggtaacggtctcgagc

SEQ ID NO: 30 - protein, 123 aa, Homo sapiens
EVQLVESGGGFVQPGGSLRLSCAVSGFPYSGTSFHWVRQASGKGLEWIGRIRSKSDNYETSYTESLKGRFTVSRDDSKNTVYLHLSSLRTEDTALYYCTTGIIVVDTSYLDHWGRGTLVTVSS

SEQ ID NO: 31 - DNA, 369 bp, Homo sapiens
  source 1..369: mol_type = other DNA
gaggtgcaactggtcgagacgggaggaggatttgtgcaaccgggggggagccttcaactatcatgcgctgtgagcggattcccctattccgggacgagctttcactgggtcagacaagcgagcggaaaagggctggaatggatcgggaggattcgaagcaagagcgacaactatgagacatcatacactgaatcactgaaggggagattcaccgtatctcgcgacgactcgaagaacacggtatacctgcaattaagctcgctgcggacggaggacacggcgctatactattgcacgacgggaattatagtcgtcgacacatcatatcttgatcattgggggcggggaaccctggtaacggtctcgagc

SEQ ID NO: 32 - protein, 123 aa, Homo sapiens
EVQLVETGGGFVQPGGSLQLSCAVSGFPYSGTSFHWVRQASGKGLEWIGRIRSKSDNYETSYTESLKGRFTVSRDDSKNTVYLQLSSLRTEDTALYYCTTGIIVVDTSYLDHWGRGTLVTVSS

SEQ ID NO: 33 - DNA, 369 bp, Homo sapiens
  source 1..369: mol_type = other DNA
gaggtgcagctggttgagactggcggaggatttgtgcaaccgggggggagcctgcggctatcatgcgcggtatcgggattcccatactctgggacaagtttccactgggtccgacaggcttcgggaaaggggctggaatggataggaaggataagatctaagagcgataactatgagacatcatacacggaatcgctgaaagggcgattcaccgtatctcgggacgatagcaagaacaccgtgagactgcaactatcaagcctacgaacggaggatacggcgctatactactgcacaaccgggataatcgtcgtcgacacatcatatttggatcattggggccgggggacgctggtaacggtctcgagc

SEQ ID NO: 34 - protein, 123 aa, Homo sapiens
EVQLVETGGGFVQPGGSLRLSCAVSGFPYSGTSFHWVRQASGKGLEWIGRIRSKSDNYETSYTESLKGRFTVSRDDSKNTVRLQLSSLRTEDTALYYCTTGIIVVDTSYLDHWGRGTLVTVSS

SEQ ID NO: 35 - DNA, 369 bp, Homo sapiens
  source 1..369: mol_type = other DNA
gaggtgcaactcgtggagaccggcgggggatttgtacaaccggggggatcgctgcggctatcatgcgccgtgagcggattcccctactcggggacatcatttcactgggtccgacaagcctccgggaaggggctggaatggattgggcggatacgatcgaagagcgacaattacgagacatcatacactgaatccctgaaagggcgatttaccgtgagccgagacgactccaagaatacggtatacctgcatttgagctcgctaaggacggaggatacggcattatactactgcacaactggaataatagtcgtcgacacgagctacttagaccactgggggaggggaacgctggtaacggtctcgagc

SEQ ID NO: 36 - protein, 123 aa, Homo sapiens
EVQLVETGGGFVQPGGSLRLSCAVSGFPYSGTSFHWVRQASGKGLEWIGRIRSKSDNYETSYTESLKGRFTVSRDDSKNTVYLHLSSLRTEDTALYYCTTGIIVVDTSYLDHWGRGTLVTVSS

SEQ ID NO: 37 - DNA, 369 bp, Homo sapiens
  source 1..369: mol_type = other DNA
gaggtgcaactggtggaatctggagggggcttcgtgcaacccggaggatcgctacaacttagctgcgccgtgagcggatttccatactcgggcacatcattccactgggtccggcaagcgagcgggaagggactggaatggatagggcggataagatcgaaatcggacaattatgagacgagctacaccgaatccctaaagggaagattcaccgtatcgagagacgattcaaagaacaccgtaagactgcaactaagctcgctgagaactgaagacactgcactatactactgcacaacggggataatagtcgtcgacacatcatatttggaccactgggggaggggaactttggtaacggtctcgagc

SEQ ID NO: 38 - protein, 123 aa, Homo sapiens
EVQLVESGGGFVQPGGSLQLSCAVSGFPYSGTSFHWVRQASGKGLEWIGRIRSKSDNYETSYTESLKGRFTVSRDDSKNTVRLQLSSLRTEDTALYYCTTGIIVVDTSYLDHWGRGTLVTVSS

SEQ ID NO: 39 - DNA, 369 bp, Homo sapiens
  source 1..369: mol_type = other DNA
gaggtgcagctggtggagagcgggggcggattcgtgcaacccggaggatcgctacaactgagctgcgccgtgagcggatttccttattcgggcacgagctttcactgggtccgacaagcgagcggaaaaggcctggaatggattgggaggatacggagcaaatccgacaattatgagacatcatacacggagagcctgaaggggagatttaccgtgagcagggacgattcgaagaatacggtatacctgcacctgagctctctgcggaccgaggacacggcgctatattattgcactacggggataatcgtcgtcgacacatcatacctggaccactgggggagggggacgctagtgacggtctcgagc

SEQ ID NO: 40 - protein, 123 aa, Homo sapiens
EVQLVESGGGFVQPGGSLQLSCAVSGFPYSGTSFHWVRQASGKGLEWIGRIRSKSDNYETSYTESLKGRFTVSRDDSKNTVYLHLSSLRTEDTALYYCTTGIIVVDTSYLDHWGRGTLVTVSS

SEQ ID NO: 41 - DNA, 369 bp, Homo sapiens
  source 1..369: mol_type = other DNA
gaggtacagctggtggaatcgggcgggggatttgtgcaaccggggggctcgctgcgcctgagctgcgcggtatccggcttcccttactctggcacatccttccattgggtccgccaagcatctgggaaaggactggaatggattgggagaatccgatcgaaatccgataactatgagacgagctataccgaatcattgaaggggcgattcaccgtgagcagggatgactctaaaaacaccgtgaggctgcatctatcgagcctacggaccgaggatacggctctatattactgcacgaccgggatcatagtcgtcgatacctcatacttggatcactgggggcggggaacattggtcacggtctcgagc

SEQ ID NO: 42 - protein, 123 aa, Homo sapiens
EVQLVESGGGFVQPGGSLRLSCAVSGFPYSGTSFHWVRQASGKGLEWIGRIRSKSDNYETSYTESLKGRFTVSRDDSKNTVRLHLSSLRTEDTALYYCTTGIIVVDTSYLDHWGRGTLVTVSS

SEQ ID NO: 43 - DNA, 369 bp, Homo sapiens
  source 1..369: mol_type = other DNA
gaggtgcaactcgtggaatcgggggggggatttgtgcaaccgggcggatcgctgcaactatcatgcgccgtgagcggatttccctactctggaacatcatttcactgggtccgacaagcgagcggaaagggattggaatggattgggcggataagatcgaagagcgataactacgagacatcatataccgaatcactgaaggggcgatttaccgtgagccgagacgactcgaagaatactgttcggctgcacctgagctcgctaaggacggaggacaccgcgctatattactgcacgaccggcataatagtcgtcgacacaagctacttggatcactgggggaggggcacgctggtaacggtctcgagc

SEQ ID NO: 44 - protein, 123 aa, Homo sapiens
EVQLVESGGGFVQPGGSLQLSCAVSGFPYSGTSFHWVRQASGKGLEWIGRIRSKSDNYETSYTESLKGRFTVSRDDSKNTVRLHLSSLRTEDTALYYCTTGIIVVDTSYLDHWGRGTLVTVSS

SEQ ID NO: 45 - DNA, 369 bp, Homo sapiens
  source 1..369: mol_type = other DNA
gaggtgcagctggtggagacgggggggggattcgtgcaaccggggggctcgctgcggctatcatgcgcggtatcgggatttccatatagcgggacatcctttcattgggtccgacaagcatctggaaaggggctggaatggattgggaggattagatcaaagagcgataattacgaaacttcatacacggaatcgctgaaagggagattcaccgtgagccgagacgactcaaagaacactgtgcgcctgcatctatcatcgctgagaaccgaggatacggcgctatattattgcaccaccgggatcattgtcgtcgacacttcatacttggaccactgggggcggggaacgcttgtgacggtctcgagc

SEQ ID NO: 46 - protein, 123 aa, Homo sapiens
EVQLVETGGGFVQPGGSLRLSCAVSGFPYSGTSFHWVRQASGKGLEWIGRIRSKSDNYETSYTESLKGRFTVSRDDSKNTVRLHLSSLRTEDTALYYCTTGIIVVDTSYLDHWGRGTLVTVSS

SEQ ID NO: 47 - DNA, 369 bp, Homo sapiens
  source 1..369: mol_type = other DNA
gaagtacagctggtggagacggggggaggatttgtgcaaccgggagggagcctgcaactatcatgcgccgtatccggcttcccatactcggggacatcattccattgggtcaggcaagcaagcggcaaagggctggaatggattgggcggattagatcaaaatccgacaattacgagacgagctacaccgaaagcctgaagggccgatttaccgtatcgcgggacgattcgaagaacacggtatacctgcaccttagctcactgaggacggaggacacggccttatactattgcacgaccgggattatcgtcgtcgacacatcatacttggatcattgggggcgaggcacactcgttaccgtctcgagc

SEQ ID NO: 48 - protein, 123 aa, Homo sapiens
EVQLVETGGGFVQPGGSLQLSCAVSGFPYSGTSFHWVRQASGKGLEWIGRIRSKSDNYETSYTESLKGRFTVSRDDSKNTVYLHLSSLRTEDTALYYCTTGIIVVDTSYLDHWGRGTLVTVSS

SEQ ID NO: 49 - DNA, 369 bp, Homo sapiens
  source 1..369: mol_type = other DNA
gaagtccaacttgtggaaactggggggggatttgtgcaaccgggagggagcctacaactgagctgcgcggtctccggcttcccctactcggggacatcctttcactgggtccgacaagcatccgggaaggggctggaatggattggacgcatacggagcaaatctgacaattacgagacatcatacactgaatcgctaaagggccgatttacggtctcgcgggacgattcgaagaataccgtccggctgcaactatcgagcctgcggaccgaggataccgcgctatattattgcaccacgggaattattgtcgtcgatactagctatctggatcactgggggagggggacgctggtcacggtctcgagc

SEQ ID NO: 50 - protein, 123 aa, Homo sapiens
EVQLVETGGGFVQPGGSLQLSCAVSGFPYSGTSFHWVRQASGKGLEWIGRIRSKSDNYETSYTESLKGRFTVSRDDSKNTVRLQLSSLRTEDTALYYCTTGIIVVDTSYLDHWGRGTLVTVSS

SEQ ID NO: 51 - DNA, 369 bp, Homo sapiens
  source 1..369: mol_type = other DNA
gaggtgcagctggtcgaatctggagggggatttgtgcaacctggcggaagtttgcggctgagctgcgccgtgagcggattcccatattcggggacgagctttcactgggtccggcaatcgagcgggaaggggcttgaatggataggacggattcggagcaaatccgacaactacgaaacatcatataccgagagcctgaaggggagattcacggtatcgagagatgattcgaagaacactgtatatctgcaactatcatcactgagaacggaggacacggcgctatattactgcacaaccggaattatagtcgtcgacacatcatacctcgaccactgggggcgaggcacgctggttacggtctcgagc

SEQ ID NO: 52 - protein, 123 aa, Homo sapiens
EVQLVESGGGFVQPGGSLRLSCAVSGFPYSGTSFHWVRQSSGKGLEWIGRIRSKSDNYETSYTESLKGRFTVSRDDSKNTVYLQLSSLRTEDTALYYCTTGIIVVDTSYLDHWGRGTLVTVSS

SEQ ID NO: 53 - DNA, 369 bp, Homo sapiens
  source 1..369: mol_type = other DNA
gaggtgcaactggtggaatccggcgggggattcgtgcaaccggggggatcgctgcgactatcatgcgccgtaagcggatttacatttagcgggacatcatttcactgggtccggcaagcaagcggaaaggggctggaatggattggacggattaggagcaaatcggataactatgagacaagctatacggaatcgctgaaagggagatttaccgtatcgcgcgatgactcgaagaacaccgtatacctgcaactatcgagcttgcggaccgaggacaccgcactatactattgcacaactggaataatcgtcgtcgacacatcatacctagaccactggggaaggggcacactggtcacggtctcgagc

SEQ ID NO: 54 - protein, 123 aa, Homo sapiens
EVQLVESGGGFVQPGGSLRLSCAVSGFTFSGTSFHWVRQASGKGLEWIGRIRSKSDNYETSYTESLKGRFTVSRDDSKNTVYLQLSSLRTEDTALYYCTTGIIVVDTSYLDHWGRGTLVTVSS

SEQ ID NO: 55 - DNA, 324 bp, Homo sapiens
  source 1..324: mol_type = other DNA
tcctatgaactgacacagcctccttccgcaagcgtatctcctgggcagaccgcacggattacatgcagtggggccgcgttgcctaaaaagtacgcctactggtatcaactgaaatcagggcaagccccagtcttagtgatttacgaggacactaagcggcctagtggcatacccgaaagattcagtggcagcagctctgggactactgcaactttgacaatcaatggtgcccaagtggaggatgaggctgactactattgttatagcactgactccagtggcgacgtctgggtgtttggaggcggtaccaagctgacagttctg

SEQ ID NO: 56 - protein, 108 aa, Homo sapiens
SYELTQPPSASVSPGQTARITCSGAALPKKYAYWYQLKSGQAPVLVIYEDTKRPSGIPERFSGSSSGTTATLTINGAQVEDEADYYCYSTDSSGDVWVFGGGTKLTVL

SEQ ID NO: 57 - DNA, 324 bp, Homo sapiens
  source 1..324: mol_type = other DNA
tcgtatgagctaacccagccacccagtgcgagcgtgtcgccaggccagaccgccagaattacctgtagcggtgctgcactacccaaaaagtacgcctattggtatcaacagaaaagcggacaggccccagtcctagttatctacgaagatactaaacgacccagcggaatccccgagcggttcagtggctcatcgtcaggaactacagctactttgacaatttctggagctcaggtcgaggacgaagctgattactactgttactccactgacagcagcggcgacgtgtgggtgttcggaggcggtaccaagctgaccgttctg

SEQ ID NO: 58 - protein, 108 aa, Homo sapiens
SYELTQPPSASVSPGQTARITCSGAALPKKYAYWYQQKSGQAPVLVIYEDTKRPSGIPERFSGSSSGTTATLTISGAQVEDEADYYCYSTDSSGDVWVFGGGTKLTVL

SEQ ID NO: 59 - DNA, 324 bp, Homo sapiens
  source 1..324: mol_type = other DNA
agctacgaactgacccaaccaccatccgcatctgttagcccaggtcaaactgcgcggatcacttgcagtggggctgcgcttccaaagaagtatgcctactggtatcaacaaaagtccggtcaagcaccagttttggttatttatgaggatacaaaaaggccatcagggataccagagagattttcagggtcttctagcgggactacggcgacacttacaatttccggcgctcaagtcgaggacgaggccgattactattgttattcgacggaatcatctggcgacgtctgggtcttcggaggcggtaccaagttgactgtttta

SEQ ID NO: 60 - protein, 108 aa, Homo sapiens
SYELTQPPSASVSPGQTARITCSGAALPKKYAYWYQQKSGQAPVLVIYEDTKRPSGIPERFSGSSSGTTATLTISGAQVEDEADYYCYSTESSGDVWVFGGGTKLTVL

SEQ ID NO: 61 - protein, 11 aa, Homo sapiens
YSTESSGDVWV

SEQ ID NO: 62 - protein, 15 aa, Homo sapiens
TPKTVTPASSAKTSP

SEQ ID NO: 63 - protein, 15 aa, Homo sapiens
VTPASSAKTSPAKQQ

SEQ ID NO: 64 - protein, 5 aa, Homo sapiens
ASSAK

SEQ ID NO: 65 - protein, 11 aa, Homo sapiens
VTPASSAKTSP

SEQ ID NO: 66 - protein, 22 aa, Homo sapiens
  SITE 11: note = Phosphorylation site
YATPAPSAKSSPSKHQPPPIRC

SEQ ID NO: 67 - protein, 22 aa, Homo sapiens
  SITE 11: note = Phosphorylation site
TVTPASSAKTSPAKQQAPPVRC

SEQ ID NO: 68 - protein, 22 aa, Homo sapiens
  SITE 11: note = Phosphorylation site
GGTPAGSARGSPTRPNPPVRNC

SEQ ID NO: 69 - protein, 24 aa, Homo sapiens
  SITE 5: note = Phosphorylation site
  SITE 10: note = Phosphorylation site
  SITE 18: note = Phosphorylation site
EVPATPKYATPAPSAKSSPSKHQC

SEQ ID NO: 70 - protein, 24 aa, Homo sapiens
  SITE 5: note = Phosphorylation site
  SITE 10: note = Phosphorylation site
  SITE 18: note = Phosphorylation site
EVSVTPKTVTPASSAKTSPAKQQC

SEQ ID NO: 71 - protein, 24 aa, Homo sapiens
  SITE 5: note = Phosphorylation site
  SITE 10: note = Phosphorylation site
  SITE 18: note = Phosphorylation site
DLTTTPKGGTPAGSARGSPTRPNC

SEQ ID NO: 72 - protein, 26 aa, Homo sapiens
  SITE 7: note = T509 phospho-site (Peptide 4152961)
  SITE 12: note = T514 phospho-site (Peptide 4152962)
  SITE 20: note = S522 phospho-site (Peptide 4152963)
VCEVSVTPKTVTPASSAKTSPAKQQA